European Patent Application EP 4 678 749 A1, published January 14, 2026. Title: Neutralizable blood clotting inhibitor. Applicant: The University of Tokyo. Application JP. The sequence listing filed with the application follows.

SEQUENCE LISTING (149 sequences)

SEQ ID NO: 1 - DNA, 15 bp, synthetic construct
  source 1..15: mol_type = other DNA
ggttggtgtggttgg

SEQ ID NO: 2 - DNA, 26 bp, synthetic construct
  source 1..26: mol_type = other DNA
cgcctaggttgggtagggtggtggcg

SEQ ID NO: 3 - DNA, 29 bp, synthetic construct
  source 1..29: mol_type = other DNA
agtccgtggtagggcaggttggggtgact

SEQ ID NO: 4 - DNA, 72 bp, synthetic construct
  source 1..72: mol_type = other DNA
aggtcagatgatggggatggggggttggaggaatggatgacctagtccgtggtagggcaggttggggtgact

SEQ ID NO: 5 - DNA, 82 bp, synthetic construct
  source 1..82: mol_type = other DNA
taaggtcagatgatggggatggggggttggaggaatggatgaccttatatagtccgtggtagggcaggttggggtgactata

SEQ ID NO: 6 - DNA, 106 bp, synthetic construct
  source 1..106: mol_type = other DNA
tatatataaggtcagatgatggggatggggggttggaggaatggatgaccttatatatatatatatatagtccgtggtagggcaggttggggtgactatatatata

SEQ ID NO: 7 - DNA, 114 bp, synthetic construct
  source 1..114: mol_type = other DNA
tatatatataaggtcagatgatggggatggggggttggaggaatggatgaccttatatatatatatatatatatagtccgtggtagggcaggttggggtgactatatatatata

SEQ ID NO: 8 - DNA, 82 bp, synthetic construct
  source 1..82: mol_type = other DNA
aaaggtcagatgatggggatggggggttggaggaatggatgacctttacgagtccgtggtagggcaggttggggtgactcgt

SEQ ID NO: 9 - DNA, 106 bp, synthetic construct
  source 1..106: mol_type = other DNA
gtcactagaggtcagatgatggggatggggggttggaggaatggatgacctctagtgactgatttacgagtccgtggtagggcaggttggggtgactcgtaaatca

SEQ ID NO: 10 - DNA, 114 bp, synthetic construct
  source 1..114: mol_type = other DNA
cactagactgaggtcagatgatggggatggggggttggaggaatggatgacctcagtctagtgactgatttacgagtccgtggtagggcaggttggggtgactcgtaaatcagt

SEQ ID NO: 11 - DNA, 89 bp, synthetic construct
  source 1..89: mol_type = other DNA
aggtcagatgatggggatggggggttggaggaatggatgaccttttttttttttttttttagtccgtggtagggcaggttggggtgact

SEQ ID NO: 12 - DNA, 120 bp, synthetic construct
  source 1..120: mol_type = other DNA
cagtcactagaggtcagatgatggggatggggggttggaggaatggatgacctctagtgactgatttacgaggtcagatggtggtcggggtggtgggatgagggttctgacctcgtaaat

SEQ ID NO: 13 - DNA, 106 bp, synthetic construct; identical to SEQ ID NO: 9
  source 1..106: mol_type = other DNA

SEQ ID NO: 14 - DNA, 43 bp, synthetic construct
  source 1..43: mol_type = other DNA
aggtcagatgatggggatggggggttggaggaatggatgacct

SEQ ID NO: 15 - DNA, 32 bp, synthetic construct
  source 1..32: mol_type = other DNA
ccccatccccatcatctgacctctagtgactg

SEQ ID NO: 16 - DNA, 22 bp, synthetic construct
  source 1..22: mol_type = other DNA
ccccatccccatcatctgacct

SEQ ID NO: 17 - DNA, 30 bp, synthetic construct
  source 1..30: mol_type = other DNA
ccccatccccatcatctgacctctagtgac

SEQ ID NO: 18 - DNA, 33 bp, synthetic construct
  source 1..33: mol_type = other DNA
agatgatggggatggggggttggaggaatggat

SEQ ID NO: 19 - DNA, 29 bp, synthetic construct
  source 1..29: mol_type = other DNA
atggtggtcggggtggtgggatgagggtt

SEQ ID NO: 20 - DNA, 23 bp, synthetic construct
  source 1..23: mol_type = other DNA
ccgtggtagggcaggttggggtg

SEQ ID NO: 21 - DNA, 43 bp, synthetic construct
  source 1..43: mol_type = other DNA
aggtcagatggtggtcggggtggtgggatgagggttctgacct

SEQ ID NO: 22 - DNA, 120 bp, synthetic construct
  source 1..120: mol_type = other DNA
gtcactagaggtcagatgatggggatggggggttggaggaatggatgacctctagtgactgatttacgaggtcagatgatggggatggggggttggaggaatggatgacctcgtaaatca

SEQ ID NO: 23 - DNA, 21 bp, synthetic construct
  source 1..21: mol_type = other DNA
aggtcagatgatggggatggg

SEQ ID NO: 24 - DNA, 17 bp, synthetic construct
  source 1..17: mol_type = other DNA
ctagtgactgatttacg

SEQ ID NO: 25 - DNA, 17 bp, synthetic construct
  source 1..17: mol_type = other DNA
cgtaaatcagtcactag

SEQ ID NO: 26 - DNA, 64 bp, synthetic construct
  source 1..64: mol_type = other DNA
gtcagatgatggggatggggggttggaggaatggatgacctagtctagtgactgatttacgagt

SEQ ID NO: 27 - DNA, 48 bp, synthetic construct
  source 1..48: mol_type = other DNA
ccgtggtagggcaggttggggtgactcgtaaatcagtcactagactag

SEQ ID NO: 28 - DNA, 61 bp, synthetic construct
  source 1..61: mol_type = other DNA
aggtcagatgatggggatggggggttggaggaatggatgacctagtctagtgactgattta

SEQ ID NO: 29 - DNA, 48 bp, synthetic construct
  source 1..48: mol_type = other DNA
gtccgtggtagggcaggttggggtgactcgtaaatcagtcactagact

SEQ ID NO: 30 - DNA, 64 bp, synthetic construct
  source 1..64: mol_type = other DNA
ctaggtcagatgatggggatggggggttggaggaatggatgacctagtctagtgactgatttac

SEQ ID NO: 31 - DNA, 48 bp, synthetic construct
  source 1..48: mol_type = other DNA
gagtccgtggtagggcaggttggggtgactcgtaaatcagtcactaga

SEQ ID NO: 32 - DNA, 64 bp, synthetic construct
  source 1..64: mol_type = other DNA
gactaggtcagatgatggggatggggggttggaggaatggatgacctagtctagtgactgattt

SEQ ID NO: 33 - DNA, 48 bp, synthetic construct
  source 1..48: mol_type = other DNA
acgagtccgtggtagggcaggttggggtgactcgtaaatcagtcacta

SEQ ID NO: 34 - DNA, 64 bp, synthetic construct
  source 1..64: mol_type = other DNA
tagactaggtcagatgatggggatggggggttggaggaatggatgacctagtctagtgactgat

SEQ ID NO: 35 - DNA, 48 bp, synthetic construct
  source 1..48: mol_type = other DNA
ttacgagtccgtggtagggcaggttggggtgactcgtaaatcagtcac

SEQ ID NO: 36 - DNA, 63 bp, synthetic construct
  source 1..63: mol_type = other DNA
gtcagatgatggggatggggggttggaggaatggatgacctgtctagtgactgatttacgagt

SEQ ID NO: 37 - DNA, 47 bp, synthetic construct
  source 1..47: mol_type = other DNA
ccgtggtagggcaggttggggtgactcgtaaatcagtcactagacag

SEQ ID NO: 38 - DNA, 63 bp, synthetic construct
  source 1..63: mol_type = other DNA
aggtcagatgatggggatggggggttggaggaatggatgacctgtctagtgactgatttacga

SEQ ID NO: 39 - DNA, 47 bp, synthetic construct
  source 1..47: mol_type = other DNA
gtccgtggtagggcaggttggggtgactcgtaaatcagtcactagac

SEQ ID NO: 40 - DNA, 63 bp, synthetic construct
  source 1..63: mol_type = other DNA
acaggtcagatgatggggatggggggttggaggaatggatgacctgtctagtgactgatttac

SEQ ID NO: 41 - DNA, 47 bp, synthetic construct
  source 1..47: mol_type = other DNA
gagtccgtggtagggcaggttggggtgactcgtaaatcagtcactag

SEQ ID NO: 42 - DNA, 63 bp, synthetic construct
  source 1..63: mol_type = other DNA
agacaggtcagatgatggggatggggggttggaggaatggatgacctgtctagtgactgattt

SEQ ID NO: 43 - DNA, 47 bp, synthetic construct
  source 1..47: mol_type = other DNA
acgagtccgtggtagggcaggttggggtgactcgtaaatcagtcact

SEQ ID NO: 44 - DNA, 63 bp, synthetic construct
  source 1..63: mol_type = other DNA
ctagacaggtcagatgatggggatggggggttggaggaatggatgacctgtctagtgactgat

SEQ ID NO: 45 - DNA, 47 bp, synthetic construct
  source 1..47: mol_type = other DNA
ttacgagtccgtggtagggcaggttggggtgactcgtaaatcagtca

SEQ ID NO: 46 - DNA, 62 bp, synthetic construct
  source 1..62: mol_type = other DNA
gtcagatgatggggatggggggttggaggaatggatgaccttctagtgactgatttacgagt

SEQ ID NO: 47 - DNA, 46 bp, synthetic construct
  source 1..46: mol_type = other DNA
ccgtggtagggcaggttggggtgactcgtaaatcagtcactagaag

SEQ ID NO: 48 - DNA, 62 bp, synthetic construct
  source 1..62: mol_type = other DNA
aggtcagatgatggggatggggggttggaggaatggatgaccttctagtgactgatttacga

SEQ ID NO: 49 - DNA, 46 bp, synthetic construct
  source 1..46: mol_type = other DNA
gtccgtggtagggcaggttggggtgactcgtaaatcagtcactaga

SEQ ID NO: 50 - DNA, 62 bp, synthetic construct
  source 1..62: mol_type = other DNA
gaaggtcagatgatggggatggggggttggaggaatggatgaccttctagtgactgatttac

SEQ ID NO: 51 - DNA, 46 bp, synthetic construct
  source 1..46: mol_type = other DNA
gagtccgtggtagggcaggttggggtgactcgtaaatcagtcacta

SEQ ID NO: 52 - DNA, 62 bp, synthetic construct
  source 1..62: mol_type = other DNA
tagaaggtcagatgatggggatggggggttggaggaatggatgaccttctagtgactgattt

SEQ ID NO: 53 - DNA, 46 bp, synthetic construct
  source 1..46: mol_type = other DNA
acgagtccgtggtagggcaggttggggtgactcgtaaatcagtcac

SEQ ID NO: 54 - DNA, 62 bp, synthetic construct
  source 1..62: mol_type = other DNA
actagaaggtcagatgatggggatggggggttggaggaatggatgaccttctagtgactgat

SEQ ID NO: 55 - DNA, 46 bp, synthetic construct
  source 1..46: mol_type = other DNA
ttacgagtccgtggtagggcaggttggggtgactcgtaaatcagtc

SEQ ID NO: 56 - DNA, 61 bp, synthetic construct
  source 1..61: mol_type = other DNA
gtcagatgatggggatggggggttggaggaatggatgacctctagtgactgatttacgagt

SEQ ID NO: 57 - DNA, 45 bp, synthetic construct
  source 1..45: mol_type = other DNA
ccgtggtagggcaggttggggtgactcgtaaatcagtcactagag

SEQ ID NO: 58 - DNA, 61 bp, synthetic construct
  source 1..61: mol_type = other DNA
aggtcagatgatggggatggggggttggaggaatggatgacctctagtgactgatttacga

SEQ ID NO: 59 - DNA, 45 bp, synthetic construct
  source 1..45: mol_type = other DNA
gtccgtggtagggcaggttggggtgactcgtaaatcagtcactag

SEQ ID NO: 60 - DNA, 61 bp, synthetic construct
  source 1..61: mol_type = other DNA
agaggtcagatgatggggatggggggttggaggaatggatgacctctagtgactgatttac

SEQ ID NO: 61 - DNA, 45 bp, synthetic construct
  source 1..45: mol_type = other DNA
gagtccgtggtagggcaggttggggtgactcgtaaatcagtcact

SEQ ID NO: 62 - DNA, 61 bp, synthetic construct
  source 1..61: mol_type = other DNA
ctagaggtcagatgatggggatggggggttggaggaatggatgacctctagtgactgattt

SEQ ID NO: 63 - DNA, 45 bp, synthetic construct
  source 1..45: mol_type = other DNA
acgagtccgtggtagggcaggttggggtgactcgtaaatcagtca

SEQ ID NO: 64 - DNA, 61 bp, synthetic construct
  source 1..61: mol_type = other DNA
cactagaggtcagatgatggggatggggggttggaggaatggatgacctctagtgactgat

SEQ ID NO: 65 - DNA, 45 bp, synthetic construct
  source 1..45: mol_type = other DNA
ttacgagtccgtggtagggcaggttggggtgactcgtaaatcagt

SEQ ID NO: 66 - DNA, 60 bp, synthetic construct
  source 1..60: mol_type = other DNA
gtcagatgatggggatggggggttggaggaatggatgaccttagtgactgatttacgagt

SEQ ID NO: 67 - DNA, 44 bp, synthetic construct
  source 1..44: mol_type = other DNA
ccgtggtagggcaggttggggtgactcgtaaatcagtcactaag

SEQ ID NO: 68 - DNA, 60 bp, synthetic construct
  source 1..60: mol_type = other DNA
aggtcagatgatggggatggggggttggaggaatggatgaccttagtgactgatttacga

SEQ ID NO: 69 - DNA, 44 bp, synthetic construct
  source 1..44: mol_type = other DNA
gtccgtggtagggcaggttggggtgactcgtaaatcagtcacta

SEQ ID NO: 70 - DNA, 60 bp, synthetic construct
  source 1..60: mol_type = other DNA
taaggtcagatgatggggatggggggttggaggaatggatgaccttagtgactgatttac

SEQ ID NO: 71 - DNA, 44 bp, synthetic construct
  source 1..44: mol_type = other DNA
gagtccgtggtagggcaggttggggtgactcgtaaatcagtcac

SEQ ID NO: 72 - DNA, 60 bp, synthetic construct
  source 1..60: mol_type = other DNA
actaaggtcagatgatggggatggggggttggaggaatggatgaccttagtgactgattt

SEQ ID NO: 73 - DNA, 44 bp, synthetic construct
  source 1..44: mol_type = other DNA
acgagtccgtggtagggcaggttggggtgactcgtaaatcagtc

SEQ ID NO: 74 - DNA, 60 bp, synthetic construct
  source 1..60: mol_type = other DNA
tcactaaggtcagatgatggggatggggggttggaggaatggatgaccttagtgactgat

SEQ ID NO: 75 - DNA, 44 bp, synthetic construct
  source 1..44: mol_type = other DNA
ttacgagtccgtggtagggcaggttggggtgactcgtaaatcag

SEQ ID NO: 76 - DNA, 59 bp, synthetic construct
  source 1..59: mol_type = other DNA
gtcagatgatggggatggggggttggaggaatggatgacctagtgactgatttacgagt

SEQ ID NO: 77 - DNA, 43 bp, synthetic construct
  source 1..43: mol_type = other DNA
ccgtggtagggcaggttggggtgactcgtaaatcagtcactag

SEQ ID NO: 78 - DNA, 59 bp, synthetic construct
  source 1..59: mol_type = other DNA
aggtcagatgatggggatggggggttggaggaatggatgacctagtgactgatttacga

SEQ ID NO: 79 - DNA, 43 bp, synthetic construct
  source 1..43: mol_type = other DNA
gtccgtggtagggcaggttggggtgactcgtaaatcagtcact

SEQ ID NO: 80 - DNA, 59 bp, synthetic construct
  source 1..59: mol_type = other DNA
ctaggtcagatgatggggatggggggttggaggaatggatgacctagtgactgatttac

SEQ ID NO: 81 - DNA, 43 bp, synthetic construct
  source 1..43: mol_type = other DNA
gagtccgtggtagggcaggttggggtgactcgtaaatcagtca

SEQ ID NO: 82 - DNA, 59 bp, synthetic construct
  source 1..59: mol_type = other DNA
cactaggtcagatgatggggatggggggttggaggaatggatgacctagtgactgattt

SEQ ID NO: 83 - DNA, 43 bp, synthetic construct
  source 1..43: mol_type = other DNA
acgagtccgtggtagggcaggttggggtgactcgtaaatcagt

SEQ ID NO: 84 - DNA, 59 bp, synthetic construct
  source 1..59: mol_type = other DNA
gtcactaggtcagatgatggggatggggggttggaggaatggatgacctagtgactgat

SEQ ID NO: 85 - DNA, 43 bp, synthetic construct
  source 1..43: mol_type = other DNA
ttacgagtccgtggtagggcaggttggggtgactcgtaaatca

SEQ ID NO: 86 - DNA, 58 bp, synthetic construct
  source 1..58: mol_type = other DNA
gtcagatgatggggatggggggttggaggaatggatgacctgtgactgatttacgagt

SEQ ID NO: 87 - DNA, 42 bp, synthetic construct
  source 1..42: mol_type = other DNA
ccgtggtagggcaggttggggtgactcgtaaatcagtcacag

SEQ ID NO: 88 - DNA, 58 bp, synthetic construct
  source 1..58: mol_type = other DNA
aggtcagatgatggggatggggggttggaggaatggatgacctgtgactgatttacga

SEQ ID NO: 89 - DNA, 42 bp, synthetic construct
  source 1..42: mol_type = other DNA
gtccgtggtagggcaggttggggtgactcgtaaatcagtcac

SEQ ID NO: 90 - DNA, 58 bp, synthetic construct
  source 1..58: mol_type = other DNA
acaggtcagatgatggggatggggggttggaggaatggatgacctgtgactgatttac

SEQ ID NO: 91 - DNA, 42 bp, synthetic construct
  source 1..42: mol_type = other DNA
gagtccgtggtagggcaggttggggtgactcgtaaatcagtc

SEQ ID NO: 92 - DNA, 58 bp, synthetic construct
  source 1..58: mol_type = other DNA
tcacaggtcagatgatggggatggggggttggaggaatggatgacctgtgactgattt

SEQ ID NO: 93 - DNA, 42 bp, synthetic construct
  source 1..42: mol_type = other DNA
acgagtccgtggtagggcaggttggggtgactcgtaaatcag

SEQ ID NO: 94 - DNA, 58 bp, synthetic construct
  source 1..58: mol_type = other DNA
agtcacaggtcagatgatggggatggggggttggaggaatggatgacctgtgactgat

SEQ ID NO: 95 - DNA, 42 bp, synthetic construct
  source 1..42: mol_type = other DNA
ttacgagtccgtggtagggcaggttggggtgactcgtaaatc

SEQ ID NO: 96 - DNA, 57 bp, synthetic construct
  source 1..57: mol_type = other DNA
gtcagatgatggggatggggggttggaggaatggatgaccttgactgatttacgagt

SEQ ID NO: 97 - DNA, 41 bp, synthetic construct
  source 1..41: mol_type = other DNA
ccgtggtagggcaggttggggtgactcgtaaatcagtcaag

SEQ ID NO: 98 - DNA, 57 bp, synthetic construct
  source 1..57: mol_type = other DNA
aggtcagatgatggggatggggggttggaggaatggatgaccttgactgatttacga

SEQ ID NO: 99 - DNA, 41 bp, synthetic construct
  source 1..41: mol_type = other DNA
gtccgtggtagggcaggttggggtgactcgtaaatcagtca

SEQ ID NO: 100 - DNA, 57 bp, synthetic construct
  source 1..57: mol_type = other DNA
caaggtcagatgatggggatggggggttggaggaatggatgaccttgactgatttac

SEQ ID NO: 101 - DNA, 41 bp, synthetic construct
  source 1..41: mol_type = other DNA
gagtccgtggtagggcaggttggggtgactcgtaaatcagt

SEQ ID NO: 102 - DNA, 57 bp, synthetic construct
  source 1..57: mol_type = other DNA
gtcaaggtcagatgatggggatggggggttggaggaatggatgaccttgactgattt

SEQ ID NO: 103 - DNA, 41 bp, synthetic construct
  source 1..41: mol_type = other DNA
acgagtccgtggtagggcaggttggggtgactcgtaaatca

SEQ ID NO: 104 - DNA, 57 bp, synthetic construct
  source 1..57: mol_type = other DNA
cagtcaaggtcagatgatggggatggggggttggaggaatggatgaccttgactgat

SEQ ID NO: 105 - DNA, 41 bp, synthetic construct
  source 1..41: mol_type = other DNA
ttacgagtccgtggtagggcaggttggggtgactcgtaaat

SEQ ID NO: 106 - DNA, 22 bp, synthetic construct
  source 1..22: mol_type = other DNA
tggggatggggggttggaggaa

SEQ ID NO: 107 - DNA, 36 bp, synthetic construct
  source 1..36: mol_type = other DNA
aggtcaatggggatggggggttggaggaattgacct

SEQ ID NO: 108 - DNA, 70 bp, synthetic construct
  source 1..70: mol_type = other DNA
aggtcaatggggatggggggttggaggaattgacctttacgagtccgtggtagggcaggttggggtgact

SEQ ID NO: 109 - DNA, 70 bp, synthetic construct
  source 1..70: mol_type = other DNA
aggtcaatggggatggggggttggaggaattgacctaaaaaagtccgtggtagggcaggttggggtgact

SEQ ID NO: 110 - DNA, 69 bp, synthetic construct
  source 1..69: mol_type = other DNA
aggtcaatggggatggggggttggaggaattgacctaaaaagtccgtggtagggcaggttggggtgact

SEQ ID NO: 111 - DNA, 67 bp, synthetic construct
  source 1..67: mol_type = other DNA
aggtcaatggggatggggggttggaggaattgacctaaagtccgtggtagggcaggttggggtgact

SEQ ID NO: 112 - DNA, 70 bp, synthetic construct
  source 1..70: mol_type = other DNA
aggtcaatggggatggggggttggaggaattgaccttttttagtccgtggtagggcaggttggggtgact

SEQ ID NO: 113 - DNA, 69 bp, synthetic construct
  source 1..69: mol_type = other DNA
aggtcaatggggatggggggttggaggaattgacctttttagtccgtggtagggcaggttggggtgact

SEQ ID NO: 114 - DNA, 67 bp, synthetic construct
  source 1..67: mol_type = other DNA
aggtcaatggggatggggggttggaggaattgacctttagtccgtggtagggcaggttggggtgact

SEQ ID NO: 115 - DNA, 65 bp, synthetic construct
  source 1..65: mol_type = other DNA
aggtcaatggggatggggggttggaggaattgacctagtccgtggtagggcaggttggggtgact

SEQ ID NO: 116 - DNA, 64 bp, synthetic construct
  source 1..64: mol_type = other DNA
taggtcaatggggatggggggttggaggaattgaccagtccgtggtagggcaggttggggtgac

SEQ ID NO: 117 - DNA, 64 bp, synthetic construct
  source 1..64: mol_type = other DNA
ctaggtcaatggggatggggggttggaggaattgaccagtccgtggtagggcaggttggggtga

SEQ ID NO: 118 - DNA, 64 bp, synthetic construct
  source 1..64: mol_type = other DNA
actaggtcaatggggatggggggttggaggaattgaccagtccgtggtagggcaggttggggtg

SEQ ID NO: 119 - DNA, 70 bp, synthetic construct
  source 1..70: mol_type = other DNA
agtccgtggtagggcaggttggggtgactcgtaaaggtcaatggggatggggggttggaggaattgacct

SEQ ID NO: 120 - DNA, 70 bp, synthetic construct
  source 1..70: mol_type = other DNA
agtccgtggtagggcaggttggggtgactaaaaaaggtcaatggggatggggggttggaggaattgacct

SEQ ID NO: 121 - DNA, 69 bp, synthetic construct
  source 1..69: mol_type = other DNA
agtccgtggtagggcaggttggggtgactaaaaaggtcaatggggatggggggttggaggaattgacct

SEQ ID NO: 122 - DNA, 67 bp, synthetic construct
  source 1..67: mol_type = other DNA
agtccgtggtagggcaggttggggtgactaaaggtcaatggggatggggggttggaggaattgacct

SEQ ID NO: 123 - DNA, 70 bp, synthetic construct
  source 1..70: mol_type = other DNA
agtccgtggtagggcaggttggggtgacttttttaggtcaatggggatggggggttggaggaattgacct

SEQ ID NO: 124 - DNA, 69 bp, synthetic construct
  source 1..69: mol_type = other DNA
agtccgtggtagggcaggttggggtgactttttaggtcaatggggatggggggttggaggaattgacct

SEQ ID NO: 125 - DNA, 67 bp, synthetic construct
  source 1..67: mol_type = other DNA
agtccgtggtagggcaggttggggtgactttaggtcaatggggatggggggttggaggaattgacct

SEQ ID NO: 126 - DNA, 65 bp, synthetic construct
  source 1..65: mol_type = other DNA
agtccgtggtagggcaggttggggtgactaggtcaatggggatggggggttggaggaattgacct

SEQ ID NO: 127 - DNA, 65 bp, synthetic construct
  source 1..65: mol_type = other DNA
gtccgtggtagggcaggttggggtgactaggtcaatggggatggggggttggaggaattgaccta

SEQ ID NO: 128 - DNA, 65 bp, synthetic construct
  source 1..65: mol_type = other DNA
tccgtggtagggcaggttggggtgactaggtcaatggggatggggggttggaggaattgacctag

SEQ ID NO: 129 - DNA, 65 bp, synthetic construct
  source 1..65: mol_type = other DNA
ccgtggtagggcaggttggggtgactaggtcaatggggatggggggttggaggaattgacctagt

SEQ ID NO: 130 - DNA, 72 bp, synthetic construct
  source 1..72: mol_type = other DNA
aggtcaatggggatggggggttggaggaattgacctaggtcaatggggatggggggttggaggaattgacct

SEQ ID NO: 131 - DNA, 68 bp, synthetic construct
  source 1..68: mol_type = other DNA
ggtcaatggggatggggggttggaggaattgaccggtcaatggggatggggggttggaggaattgacc

SEQ ID NO: 132 - DNA, 64 bp, synthetic construct
  source 1..64: mol_type = other DNA
gtcaatggggatggggggttggaggaattgacgtcaatggggatggggggttggaggaattgac

SEQ ID NO: 133 - DNA, 60 bp, synthetic construct
  source 1..60: mol_type = other DNA
tcaatggggatggggggttggaggaattgatcaatggggatggggggttggaggaattga

SEQ ID NO: 134 - DNA, 72 bp, synthetic construct
  source 1..72: mol_type = other DNA
cggtcaatggggatggggggttggaggaattgaccgcggtcaatggggatggggggttggaggaattgaccg

SEQ ID NO: 135 - DNA, 60 bp, synthetic construct
  source 1..60: mol_type = other DNA
gcaatggggatggggggttggaggaattgcgcaatggggatggggggttggaggaattgc

SEQ ID NO: 136 - DNA, 72 bp, synthetic construct; identical to SEQ ID NO: 130
  source 1..72: mol_type = other DNA

SEQ ID NO: 137 - DNA, 68 bp, synthetic construct; identical to SEQ ID NO: 131
  source 1..68: mol_type = other DNA

SEQ ID NO: 138 - DNA, 64 bp, synthetic construct; identical to SEQ ID NO: 132
  source 1..64: mol_type = other DNA

SEQ ID NO: 139 - DNA, 60 bp, synthetic construct; identical to SEQ ID NO: 133
  source 1..60: mol_type = other DNA

SEQ ID NO: 140 - DNA, 72 bp, synthetic construct; identical to SEQ ID NO: 134
  source 1..72: mol_type = other DNA

SEQ ID NO: 141 - DNA, 60 bp, synthetic construct; identical to SEQ ID NO: 135
  source 1..60: mol_type = other DNA

SEQ ID NO: 142 - DNA, 36 bp, synthetic construct
  source 1..36: mol_type = other DNA
aggtcaattcctccaaccccccatccccattgacct

SEQ ID NO: 143 - DNA, 30 bp, synthetic construct
  source 1..30: mol_type = other DNA
tcaattcctccaaccccccatccccattga

SEQ ID NO: 144 - DNA, 24 bp, synthetic construct
  source 1..24: mol_type = other DNA
attcctccaaccccccatccccat

SEQ ID NO: 145 - DNA, 18 bp, synthetic construct
  source 1..18: mol_type = other DNA
cctccaaccccccatccc

SEQ ID NO: 146 - DNA, 18 bp, synthetic construct
  source 1..18: mol_type = other DNA
attcctccaaccccccat

SEQ ID NO: 147 - DNA, 18 bp, synthetic construct
  source 1..18: mol_type = other DNA
ccaaccccccatccccat

SEQ ID NO: 148 - DNA, 12 bp, synthetic construct
  source 1..12: mol_type = other DNA
ccaaccccccat

SEQ ID NO: 149 - DNA, 44 bp, synthetic construct
  source 1..44: mol_type = other DNA
ccaaccccccatccccattgacgtcaattcctccaaccccccat